European Patent Specification EP 3 559 244 B1, published November 12, 2025. Title: Plants with shortened time to flowering. Applicant: Philip Morris Products S.A. Application EP16205377.1. The sequence listing filed with the application follows.

SEQUENCE LISTING (41 sequences)

SEQ ID NO: 1 - DNA, 3539 bp, Nicotiana tabacum
tgtttattgtacattttgaactgcatcgagctgcacgattgacagatctagtctgcaacagagtactttggtttctaattatagtaatcctaacacctcagaaatttccaaaattggaattatgggtgcaaatcatctttatatatactctcaaatgacttctcagatcttacggtcactaattgtctgtaaattaagtatggtggagttcactttatatactctgagcggtgtgcccatcctcctccatcagaatatcacttaaaacaattaacgtactttataatctttccctattgtttacacacaatttaggaaagtttctaacaaagataagcccatatttcaagattagtgtcttaggattaccctaaatgaaaaaagcaatagattccctggcaatatgtttacttatattttgaatttttgcaaaaaaaataaataaatgtgtgtcaacttgcttagttgggaccacatgcaaaaactaattcaaggatttcatctgataattttatagtggagaggaaaaggcttggattaatttaagtacttattatgtagggcaaatatcacttttagcctgcggccaccatatttatattcaagccgtaaaagtgtataaaatttgtatttttttatatataatatacggaaatgtgtgtatatatatatatatatatatatatatatatatataagaaatataaaaaaaattggctattatttttcagagcagctatacaatatcattttccatatcaggtaagctgaacaacaaatcatggaccaattcgaagagcaccagtcaggtgtgaaagagaactgacatgatagcataaaatacatatcactaactcctccacatctaagagcatacatttaatttcctatatggaagataagattaattagaaaagtgtttgataaagctaagatatgttagtaccagtttgtagtatccagttgaaattttagtgtcaacttaaggataattttactatgattagaagacagttatacattcacaaagtttctgaaaggaacttataagtcttctttttattgtacttacatttgtcaagtcatatatagtacatatgacccctcctaaaggaaaagaaagtagggaaagtaccaagctagggcatatttaaaggaaaataaaatggcaattttaagatgttagagtaagggcaggggtaggccaaagaagtattggggagaagtgattagacaagacatgccactgcttcacctaaccgcggacataactagcgataggaagatgtggaggtcgagaattaaggttgtgagttgacaggtagttatgagtttactagtaatactagtactattcttgtattcttttattcttagttttttattactttgttatgtcactcgcttccattactagttatctgttgttattgcttgttgctttatttttaccatttttttagccgagggtctatcaaaaacagtctctctgcctttataggataggggtaaggctgcgtacacactaccctttccagaccccacgtatgggattaatccgagtttgttgttgttgttgttgttgatgttgttgttgttgaaaaggaaacgtttataattaagtacatgtattaagatttcattattttcggggaagaatttcgaatgtatttaaaccataaaacgtcattctcctgcaagtatttttggtgatcaagataagtatagttaaaaattgagcaatcttctttgcctacgatgtcctgtataaaactaacaaagaaaaaattcagtttatttttcaggggtagggttactttttttttaaaaaatattctatttgaagttccataaaatcccattttttatttgcaactatattgagtagatgttccgagacagcaactataagtgaggctctatttcactgttcaaccaaaatctctcacaagctaagttccttgcaatccaaaagatctctctctctctctctctctctaatggcaaggaatgtagagcctctagtagtagggagagtagtaggggatgttcttgattcatttagtcccacagttaaaatgacagtcacttacaacaataaacaagtttgcaatggccaagagctcttcccttctgcagtcactattagacctagggttgaagttcaaggtggtgatatgagaactttcttcacattggtaacttttctaattttccttcaggttattaacttttcattgctatatagacatctttcaaacctgtctagaagattcttttcttgagctgagggttcggagacagcctctctatcccacacaagataaggttaacgtctgcatataccttgccgtcccctgacaccacatatgggattatactgcgtatgttgttgttgttgtattgctatatagacatctttgataaatcactaatcatgcatgatattattcttcttattgtaggtcatcacagatcctgatgtacctggccctagtgatccgtatctgagagaacatgttcactggtatgtactacattcaagaaaatctatggaaaaaaaataactagaagagatgagtccaaaagaaaggagattaattattgtttgatttgtattttttatttgcattagattaagtcatgcaattacctagtaataaattcgttataaggacatacacaaaaggtatgctcaacataattaaagaaagaaaagcataagcattatattcttatatgcaagctcccaatctgattgtggcgaagctaagaatttcttcgggtgtttaaatttaaaagaagtgaaaaaaaatccgataaaaaatttatgtgttatatacctctaaaacttaatattgtacctatatacatattgtaatttttcgacgaatgaccactcttattgcccatgctgccaatgccaatatgtaaaatacttcgccaatagacaaatatgtatcacattaattagttacctaaataggtaattatccataataagtgggactcgtaacttgaaaaatatggttagtaatttgctacaacatgttaagatacagtgagaatgtaaatgtatatatgtcctttcacgccgtcgtaagtttatataagttaaatctggttaacaatgtaggtcatcataacactcacaattgggaataataactcttaatcatacttctttacattcatatttgcaggatagtgactgatattccaggaactacagatgccacctttggtaaattggctattttggtttcttttattaagctggtgtttgacatgctagaattaatgtactttaattttgagcaggaaaagagttggttagctatgagatcccaaggcctaatattggaatacataggtttgtgtttgttctctttaagcagaaatgcagacaatcagtcagcccacctacttcaagggatcatttcaacactcgcaactttgccaacgtaaatgaccttggtccgcctgtcgccgccgtcttcttcaatgcacaacgagagaccgccgccaggaggcgctaa

SEQ ID NO: 2 - DNA, 1539 bp, Nicotiana tabacum
atggcaaggaatgtagagcctctagtagtagggagagtagtaggggatgttcttgattcatttagtcccacagttaaaatgacagtcacttacaacaataaacaagtttgcaatggccaagagctcttcccttctgcagtcactattagacctagggttgaagttcaaggtggtgatatgagaactttcttcacattggtaacttttctaattttccttcaggttattaacttttcattgctatatagacatctttcaaacctgtctagaagattcttttcttgagctgagggttcggagacagcctctctatcccacacaagataaggttaacgtctgcatataccttgccgtcccctgacaccacatatgggattatactgcgtatgttgttgttgttgtattgctatatagacatctttgataaatcactaatcatgcatgatattattcttcttattgtaggtcatcacagatcctgatgtacctggccctagtgatccgtatctgagagaacatgttcactggtatgtactacattcaagaaaatctatggaaaaaaaataactagaagagatgagtccaaaagaaaggagattaattattgtttgatttgtattttttatttgcattagattaagtcatgcaattacctagtaataaattcgttataaggacatacacaaaaggtatgctcaacataattaaagaaagaaaagcataagcattatattcttatatgcaagctcccaatctgattgtggcgaagctaagaatttcttcgggtgtttaaatttaaaagaagtgaaaaaaaatccgataaaaaatttatgtgttatatacctctaaaacttaatattgtacctatatacatattgtaatttttcgacgaatgaccactcttattgcccatgctgccaatgccaatatgtaaaatacttcgccaatagacaaatatgtatcacattaattagttacctaaataggtaattatccataataagtgggactcgtaacttgaaaaatatggttagtaatttgctacaacatgttaagatacagtgagaatgtaaatgtatatatgtcctttcacgccgtcgtaagtttatataagttaaatctggttaacaatgtaggtcatcataacactcacaattgggaataataactcttaatcatacttctttacattcatatttgcaggatagtgactgatattccaggaactacagatgccacctttggtaaattggctattttggtttcttttattaagctggtgtttgacatgctagaattaatgtactttaattttgagcaggaaaagagttggttagctatgagatcccaaggcctaatattggaatacataggtttgtgtttgttctctttaagcagaaatgcagacaatcagtcagcccacctacttcaagggatcatttcaacactcgcaactttgccaacgtaaatgaccttggtccgcctgtcgccgccgtcttcttcaatgcacaacgagagaccgccgccaggaggcgctaa

SEQ ID NO: 3 - protein, 172 aa, Nicotiana tabacum
MARNVEPLVVGRVVGDVLDSFSPTVKMTVTYNNKQVCNGQELFPSAVTIRPRVEVQGGDMRTFFTLVITDPDVPGPSDPYLREHVHWIVTDIPGTTDATFGKELVSYEIPRPNIGIHRFVFVLFKQKCRQSVSPPTSRDHFNTRNFANVNDLGPPVAAVFFNAQRETAARRR

SEQ ID NO: 4 - DNA, 4283 bp, Nicotiana tabacum
ttcgagtcgtgataagtgttttgcaaaaatataagataagactgcatgcgtacaatagactcttttggtccggcccttttctggaccctgcgcataacggaagcttagtgcacccggcaaccgtttttcaacgttccagatgcaagaatattataaggaggctttttgacacttttaaatttaatctaatagagtttaagtttcatgcatcgactgtcaaaaaaatatttatataatcactaatacgataattacaagtgaaatgctatactaaacattaagtagtaacctaataaaacggtagctagctaatctactatatatcacgtagtattaaaattacacttatgtaaaaatctttacggtgttaagaataacttaaaagcaatttagtaatacattaatgagtgaaaaaggtgaagaggaaacgtggtgtgttttgaactgcatcgagctgcacgattgacagagctagtctggaacagagtactttggtttctaattatagtaatcctaacatctcagaaatttccataataggaattatgggtgcaaatcatctttatatatactctcaaattaatgacttctcagcaagtactgtcattgtctgtaaattaagtatggtggagttcactttatactctgagcagtgtgcccatcctcctccatcacttaaaacaattaatgtactttataatctttccctattgtttacacacacaatttaggaaagtttttaacaaagacaagcccatgtttcaagatttgtttcttaggattaccctaaatgaaaaaagcaatagattccctggcaatttacttatattttgaatttttgcaaaaacaaaaagaaaaagtgacaacttgcttagttgggaccacatgcaaaaactaatttaaggaattcatctgatatttttatagtggagaggaaaagggctggattaatttaaatattccttatttgccaaaattatttatattcgatagctgtaaaaatatataaaatttgtatatttgtttttgtatagtatacacggaaatgtatatatatacaagaaattaaaaaaaaactattattttcagagcagttatacaatattattttccctatcatgtaagcttagcttatcaacaaatcatggaccaattctaagagctccattcaggtgtgaaagagagctgacatgatagtataaaatacacatcactaactcctccacatttgagagctatagattaatttcctatatggaagataagattaattagaaaagtgtttgaataagctaagatgtgttagtaccagtttgtaatatcaagctaaaattttagtgtcaatttaaggataattttactatgattagaagacaagttatcattcacaaatttctgaaaggaacttataagactttttatttttattttttattgtacttacatttgtcaattaagtacatgtgacccctcctaaaggaaaagaaagtagggaaattaaagtaccaagttagcgcatacttaaagccaaggtaagcaaaatggcaattttaaggtgttgtagaggaaacgtttataattaagtacacgtactaagatttcattattttcgtggaagaaatttagaatgtatttaaaccataaaacgtcattctcgtgcaagtatttttggtgatcaagataagtatagttaacgttgaacaatcttctttgcttactatgtcttgtataaaactaacaaagaaaaattcagtttatttttcaggggtagggttacttttttaaaaaaaaatattctatttgaagttccataagatcccatttttaatttgtaactatattgagtagatattccaagacagcaactataaatgaggatctatttcaccgttcaatcaaaatctctcacaagctaagttcctagcaatccaaaaaagatctctctctctctctctctctctctctctctctctctctctctctctctctctctctctctaatggcaaggaatgtagagcctctagttgtagggagagtagtaggggatgttcttgattcattcagtcccaaagttaaaatgacagtcacttacaacaataaacaagtttgcaatggccaagagctcttcccttctgcggtcaccattagacctagggttgaggttcaaggtggtgatatgagaactttcttcacattggtaacttttctaaattctccttaaggttattaacttttcatttctatatagacacatcgagggtcaacagagacaactctatctcacacaaggtaggggtaaggtattcgtataccctacccggcccacatgtgagatcacactgaatatgttgttgttgtcgcatttaggggtgtacaaatgaaactgacaaactgcaccaatctgataatccgagtcaaatcgagaaaaaatccgattatggtttggtttgatttggtttggtgatggaaaaaaccccgacatatttggttttgtttggttttaactaaaaaaagtcaaaccgaaaccaaaccaaccagacattatatgtgtagaaattttaaatatatttaatacataaaaatatttatggtagtgtaatttataaatatttcttaagatttttcatagtttatcttttaacgtattatttcaaacttgggcttataatttttggatgctccaataagttttatagtccataaatgttagtaactcaaataaatcctaaaccaaaatcaaatcaatactaatgctaataaaagacattcaattcaattgtactatgaatgaaaatagtgttggatatatatttttatagtttttccacggtttagataaaatgtataacttatttttctttgagtatggttagtcatgtaaataatcttattaatcataattttaaattatgtttatttttattatggcttattaataatatttaattttttgtgcaattttattatctttattgttgaatattttagtacaatgccacgactcatctcatatttatgttattttattgaaaaacacctcatatagttctgcctcattaggattaaaaaaatatttggagcacaaattttactttttgtgttatgaagactttatgaaaaaaaaataaaataaaaacccgaaaacccgaaacctcgagaaaaatcgagattaaaaatccgacttttattggtttggtttggtatttagatttaataacccgatacaattagtttggtttggtaattagaaaatccgaatcaaacccctaaccgtgtacacccctagtcgtattggtatatagacatctttgataaatcattaatcatgcatgatattcttcgatctccttattgtaggtcatgacagaccctgatgttcctggccctagtgatccgtatctgagagaacatcttcactggtatgcactatattcaagaaaagctatggaaaaaaataactagatgagataggtaaaaaagaaaggagtttaatgattgtttgatttgcattaattatattaagtcatgccattatctagtaataaactggttataaggacatacacaaaaggtatggtcaacatataatcaaagaaagaaaagcataagcatccttatgcaagctgccaatgtcatgtaaaatacttcgctaatagacaaatatatattacattagttacctaaaagataggtatataatcagtgggactcctaacttaaaaaataaggttagtaatctgctataacgatacactgagaatcgtcgtcgtcagtttataagttaaaaattaatgtaggtcatcacaacactcacaaagagtgcctcaattgggaagagtatgttatatagttagaatttatgttacatatggaaccacagtactacagaaggataactcttaaacatacttctttaccatcatatttgcaggatagtgactgatattccaggaacaacagatgccacctttggtaagctcactattttggcattttcatttttccttcaatttcttttagtatatagctaggttggtttttgacatgctaattttgagcaggaaaagagttggttagctatgagatcccacggcctaatattggaatacataggtttgtgtttgttctgtttaagcagaaatgcagacagtcagttagtccacatgatgtttccagagatcacttcaacactcgcaactttgccaacgtaaacgatcttggcccgcctgtcgccgccgtcttcttcaatgcacaacgagagaccgccgccaggagacgctaa

SEQ ID NO: 5 - DNA, 2283 bp, Nicotiana tabacum
atggcaaggaatgtagagcctctagttgtagggagagtagtaggggatgttcttgattcattcagtcccaaagttaaaatgacagtcacttacaacaataaacaagtttgcaatggccaagagctcttcccttctgcggtcaccattagacctagggttgaggttcaaggtggtgatatgagaactttcttcacattggtaacttttctaaattctccttaaggttattaacttttcatttctatatagacacatcgagggtcaacagagacaactctatctcacacaaggtaggggtaaggtattcgtataccctacccggcccacatgtgagatcacactgaatatgttgttgttgtcgcatttaggggtgtacaaatgaaactgacaaactgcaccaatctgataatccgagtcaaatcgagaaaaaatccgattatggtttggtttgatttggtttggtgatggaaaaaaccccgacatatttggttttgtttggttttaactaaaaaaagtcaaaccgaaaccaaaccaaccagacattatatgtgtagaaattttaaatatatttaatacataaaaatatttatggtagtgtaatttataaatatttcttaagatttttcatagtttatcttttaacgtattatttcaaacttgggcttataatttttggatgctccaataagttttatagtccataaatgttagtaactcaaataaatcctaaaccaaaatcaaatcaatactaatgctaataaaagacattcaattcaattgtactatgaatgaaaatagtgttggatatatatttttatagtttttccacggtttagataaaatgtataacttatttttctttgagtatggttagtcatgtaaataatcttattaatcataattttaaattatgtttatttttattatggcttattaataatatttaattttttgtgcaattttattatctttattgttgaatattttagtacaatgccacgactcatctcatatttatgttattttattgaaaaacacctcatatagttctgcctcattaggattaaaaaaatatttggagcacaaattttactttttgtgttatgaagactttatgaaaaaaaaataaaataaaaacccgaaaacccgaaacctcgagaaaaatcgagattaaaaatccgacttttattggtttggtttggtatttagatttaataacccgatacaattagtttggtttggtaattagaaaatccgaatcaaacccctaaccgtgtacacccctagtcgtattggtatatagacatctttgataaatcattaatcatgcatgatattcttcgatctccttattgtaggtcatgacagaccctgatgttcctggccctagtgatccgtatctgagagaacatcttcactggtatgcactatattcaagaaaagctatggaaaaaaataactagatgagataggtaaaaaagaaaggagtttaatgattgtttgatttgcattaattatattaagtcatgccattatctagtaataaactggttataaggacatacacaaaaggtatggtcaacatataatcaaagaaagaaaagcataagcatccttatgcaagctgccaatgtcatgtaaaatacttcgctaatagacaaatatatattacattagttacctaaaagataggtatataatcagtgggactcctaacttaaaaaataaggttagtaatctgctataacgatacactgagaatcgtcgtcgtcagtttataagttaaaaattaatgtaggtcatcacaacactcacaaagagtgcctcaattgggaagagtatgttatatagttagaatttatgttacatatggaaccacagtactacagaaggataactcttaaacatacttctttaccatcatatttgcaggatagtgactgatattccaggaacaacagatgccacctttggtaagctcactattttggcattttcatttttccttcaatttcttttagtatatagctaggttggtttttgacatgctaattttgagcaggaaaagagttggttagctatgagatcccacggcctaatattggaatacataggtttgtgtttgttctgtttaagcagaaatgcagacagtcagttagtccacatgatgtttccagagatcacttcaacactcgcaactttgccaacgtaaacgatcttggcccgcctgtcgccgccgtcttcttcaatgcacaacgagagaccgccgccaggagacgctaa

SEQ ID NO: 6 - protein, 173 aa, Nicotiana tabacum
MARNVEPLVVGRVVGDVLDSFSPKVKMTVTYNNKQVCNGQELFPSAVTIRPRVEVQGGDMRTFFTLVMTDPDVPGPSDPYLREHLHWIVTDIPGTTDATFGKELVSYEIPRPNIGIHRFVFVLFKQKCRQSVSPHDVSRDHFNTRNFANVNDLGPPVAAVFFNAQRETAARRR

SEQ ID NO: 7 - DNA, 4296 bp, Nicotiana tabacum
catgaccttttagctactcttaactcttctgattgttctgctgtaacttgtccccttgagttaaatgtaaagttaaaggctaaagaaggggatcctctccctaatcctgaaaattatagaggcctcgttggtaagctaaatttcctcactcacactaggcctgacataagttttgttgtgcaacatcttagtcagttcatgcaacagccctgctttcctcacatgaaggcagctttgcacctgttgaggtatctcagagacacttctaattttggcctcttatactcgaattctactgatctctctttgcaggcttattgtgatagtgattggggatcctgccctgataactggagatttgtttctgatttctgtttattctttggtggcagtctcattgggtggaaatctaagaaacatgcagtggtctctttatcttcggctgaagttgagtatagatctatgagcaaggctgtggctgaaattacttgggtgtgtaggcgtctatctgatcttggggtctcttctgcttctcttgttcctctccattgtgacagtatctctgccattcacattgcctacaatcctgtcttctatgagcggaccaaagacattgagttggattgccattttgaacgtaccaagcttgctgaaggtctcatcagtttatctcacatttccagtgcttctcagctcgcgaatgtcttcatcaaacccctgtgtgggccttctcaccatcttcatattcgaaagttgggagttctctcaccctcctacttgagggggggctgttgagataggctgaaatcagtgtggctcagacccaattattatttatttatgtacatcagattaggcccattagttagtctttagttagtcttttatttctttacatatattgggccatgtatacatacatagagacccgattttgtaatagttagatgattcatttttcggttcttaatcaataagaaatatctcgaactttctctctatctctctttaaccctaaattcttcttcgttgaatctacgagaatgatgaacattaacattagaaaatgtagatttgatcaaatcttcttaatcttttgtttatcatcttttctaattgttttgtatctgattgtatattagttaaccaccaaaattgctcaaacaatctggcttcaaatttatctaacgtttgaatatatatatatggttgaaacatgaaaaataaatttttgaagatgagatgaaaaataatttttgaaagttaaaattgtatttgaacacgtattttacttgaaaagaatttgaaattttgtgagcagaaaacttaaaaaattactctaaaacttttttttgagatttgaggattttattttcaaaattttccataaaatggcttaaatctataagcaaaagatatttgaaaataattttttttttaaaaaagctctcaaattttacagccaaacggaagcttaggataaaaaagggggaaatgggggagatgggtgggcaggttgggctgaagagaaatagacaacagtgcattaacatgtcaaatcatctttatccctctttctaaaccttacaaggagtactttttattttcttttttctttttttggccctaataaaaattaaaacacatattctctagctgctaagctataactttaactcattggcaccacgacgagtaggagaataacctttttgggcttttcttttcttttctttggtcccctttttttgaactatcaatattttagtccaaacacacctgactctacagtgatctgatggccactataaatattggctttttgcaactctcttctcaccaaaatacaaatcggttgaactcttcatatataatattcccactactattactcttaactttaaatagatttcttatatatgggttcaaaaatgtctgatccccttgtgattggtagagtgattggggaagttgttgattatttcactccaagtgttaagatgtctgttacttataacagcagcaagcatgtttataatgggcatgaactctttccttcctcagtcacctctaaacctagggttgaagttcatggaggtgatttgagatctttctttacaatggtacatactgcttccttcgattttcaatacttttattaggggtggagcttagcggcggagccaagattttaactaaggggagtcaaaatataaataagtaagcacacaaaaaaatcaagggggtcaacgtatagtatatacacataaaattaagaatttaacatatttataccgtgtaattttccagcgaaggggtgtcaattgactctccttgccaatgagtggctccgccactggcggagctagagttctagttacggttcgttgtattgtgttaagaagtccacttatactgtcttttctagaatttagaattcataaattcaaaattatggctctgcccttaaatttatttttatacatttctattatatagtaaatcgtttatattgaccccttatttttcttttttaccttaattgacagatcatgatagacccagatgttcctggtcctagtgatccatatctcagggaacacctacactggtaaagaaataagttttttaattactaactcattcaattttatcgtcccttcttttccttgtttacttggagggaaaataatacgatctcatcgaaaagataaaaattcttcaggcttgttatctaaaaacttgttaaaaaataccgtaatgaaaagacatatgagtttgttattaggtatttgactaaatatgatcgatcatatggtgttcggacaagaaatattttgtgaaaaggtccgcatacttttaaaaaaagaaaatctgccttgactcttgagtttgtgcttctcgggaaaacaatttcttccttctttttttttttttttttggtttattgacctttacatattaaagacaccactgagacacatatctagaaaaattgtatttgggaacgcaaaagcaaagaaaacatgtgttattaatcttatgtcaatgccaccagcagctcaggaaaaatatggtcgatatattgtgatttgcttgcaaaaggagcaaagaagaaatcttttgataatgtttgttatgacgatgtacttaaagcaaataagttagaggtcgtttggtacatgggataaggataataattttgggataaagtttaggattaactttatcttatatttggtttggagtattagctaaccgcgaggtatttttcaaactaaaatagtgggattagctatcccatataaaaagtaggatagctaatcccatgggatatcccaccctatcggatagtaatagtccaataggagacaactctaatttgtacagacataatgtccagtcacaccttgtttttttgtcatgacacatattaagcatgaataataatatttcgacaatcttgtagcatttgattagacttagcaaattataaatatgtccaataattggtcacattgttctaataattacttgtttcccttatcattatatatagtgcttcattcactaaacagaacccaaaaaaaaaaaaaaaaaaactgcaaaatggtcatatcatgtagtaacggaataaaaacgtactcagttttatgataaaatcaaagtgacatatttgtacgctttgatagttgacaaatacctgaaaaaagaatttgaccatctttacaggattgtcacagacattccaggcactacagattgctcgtttggtatgtatctttaacccaaatttcaagcttcgaaatagtaacagcttttgtttttaatattttatttgtcttaaatacatattttccttattataaatttcttcgcctagtggtaacgggatcaggtattgattcgtatttattttttattgatcaacaaaaaaagagtacaaaagaaagaattgtttttctacacttagatttatatatatgcaatgtctagaaattaatgagtttacaaattcattgatgtgtatatctcacaatcaaatccaaaatactgatccaaaaattttgatcagggaaagaaatagttggctatgaaatgccaaggccaaatattggaattcacaggtttgtatttctgctgttcaagcagaagaagaggcaaacagtattgactgcacctctctccagggatcgatttaatacgcgtaaattcgcagaagaaaatgagcttgggtctcctgttgcagcagttttcttcaattgccagagggaaactgctgccagaaggcgttga

SEQ ID NO: 8 - DNA, 2296 bp, Nicotiana tabacum
atgtctgttacttataacagcagcaagcatgtttataatgggcatgaactctttccttcctcagtcacctctaaacctagggttgaagttcatggaggtgatttgagatctttctttacaatggtacatactgcttccttcgattttcaatacttttattaggggtggagcttagcggcggagccaagattttaactaaggggagtcaaaatataaataagtaagcacacaaaaaaatcaagggggtcaacgtatagtatatacacataaaattaagaatttaacatatttataccgtgtaattttccagcgaaggggtgtcaattgactctccttgccaatgagtggctccgccactggcggagctagagttctagttacggttcgttgtattgtgttaagaagtccacttatactgtcttttctagaatttagaattcataaattcaaaattatggctctgcccttaaatttatttttatacatttctattatatagtaaatcgtttatattgaccccttatttttcttttttaccttaattgacagatcatgatagacccagatgttcctggtcctagtgatccatatctcagggaacacctacactggtaaagaaataagttttttaattactaactcattcaattttatcgtcccttcttttccttgtttacttggagggaaaataatacgatctcatcgaaaagataaaaattcttcaggcttgttatctaaaaacttgttaaaaaataccgtaatgaaaagacatatgagtttgttattaggtatttgactaaatatgatcgatcatatggtgttcggacaagaaatattttgtgaaaaggtccgcatacttttaaaaaaagaaaatctgccttgactcttgagtttgtgcttctcgggaaaacaatttcttccttctttttttttttttttttggtttattgacctttacatattaaagacaccactgagacacatatctagaaaaattgtatttgggaacgcaaaagcaaagaaaacatgtgttattaatcttatgtcaatgccaccagcagctcaggaaaaatatggtcgatatattgtgatttgcttgcaaaaggagcaaagaagaaatcttttgataatgtttgttatgacgatgtacttaaagcaaataagttagaggtcgtttggtacatgggataaggataataattttgggataaagtttaggattaactttatcttatatttggtttggagtattagctaaccgcgaggtatttttcaaactaaaatagtgggattagctatcccatataaaaagtaggatagctaatcccatgggatatcccaccctatcggatagtaatagtccaataggagacaactctaatttgtacagacataatgtccagtcacaccttgtttttttgtcatgacacatattaagcatgaataataatatttcgacaatcttgtagcatttgattagacttagcaaattataaatatgtccaataattggtcacattgttctaataattacttgtttcccttatcattatatatagtgcttcattcactaaacagaacccaaaaaaaaaaaaaaaaaaactgcaaaatggtcatatcatgtagtaacggaataaaaacgtactcagttttatgataaaatcaaagtgacatatttgtacgctttgatagttgacaaatacctgaaaaaagaatttgaccatctttacaggattgtcacagacattccaggcactacagattgctcgtttggtatgtatctttaacccaaatttcaagcttcgaaatagtaacagcttttgtttttaatattttatttgtcttaaatacatattttccttattataaatttcttcgcctagtggtaacgggatcaggtattgattcgtatttattttttattgatcaacaaaaaaagagtacaaaagaaagaattgtttttctacacttagatttatatatatgcaatgtctagaaattaatgagtttacaaattcattgatgtgtatatctcacaatcaaatccaaaatactgatccaaaaattttgatcagggaaagaaatagttggctatgaaatgccaaggccaaatattggaattcacaggtttgtatttctgctgttcaagcagaagaagaggcaaacagtattgactgcacctctctccagggatcgatttaatacgcgtaaattcgcagaagaaaatgagcttgggtctcctgttgcagcagttttcttcaattgccagagggaaactgctgccagaaggcgttga

SEQ ID NO: 9 - protein, 148 aa, Nicotiana tabacum
MSVTYNSSKHVYNGHELFPSSVTSKPRVEVHGGDLRSFFTMIMIDPDVPGPSDPYLREHLHWIVTDIPGTTDCSFGKEIVGYEMPRPNIGIHRFVFLLFKQKKRQTVLTAPLSRDRFNTRKFAEENELGSPVAAVFFNCQRETAARRR

SEQ ID NO: 10 - DNA, 4080 bp, Nicotiana tabacum
agggcacgaccctaagaccttcttcatagctataaatagtgagctcaggtttcattgtaaatggaacgactattctggcaaacttatacaatattttatacaaaactcaattcaatcttatcttctgatttctagattctttttgtttttgtgcccgaaaaccttgttcctggaattgttgcttctgttgtttcgtccatatcttaaggctaagtgttatataattcttcaattatttatttatttatttcaggttcaaattaattcacttatctaaaaatcatgtataaatttaattgtaccattttacgggtgaacagtttggcgcccatcgtggggcctagataaccgtgtaactaaaggacaaacgtcttttcgggaacttttctattttcaagaactcaaacccgagatttagacctctgagggatctgatcatctcactacatcgctgagtggtagttgattccatatacgattaacctagtttacaactaaattaaattatgtgcattaatccaagcaacttttgatgatcagctgatcaacctaacgtaagaaagcaattaatttagatgcatatattctacaaatggaaattagtaggagcaagcaagttatgcaaaagaaaggaaaagagaaaacattagaagtaggccaaagaaagaagaaggaagaggaagcaatcagccactgttctagaatggaatatggagaaaaataataaattaaattcagatttctataagtagtaatcctcttctttctattaccggttaaagctgcagaaattttctttttcttgacatgacctgaccatagcttccaccattgtttgcaggctggtggtggagtccctttataccctcatctctcctacctaagaaccataggattaggtgattcaagtttttatttttaacaaaaaatgaaaaatttatgaaggaagttcaactttttattaccttaaataaaaaagaccttgatgctttaagtagctccaagacggtagctgcaaattccatctgcttttcctttttaataaaataatgtactacctactatctgaaagtttaacttctatgattctgtaggttttgtaaaacacttgggggtatttatattttataggggattgcaattagaggcagatacaatttggtttagttaaccaccgatattactcaaacaatttggctttaaatctggttagtgtttggatatagatttggttgaaatttgaagaaaaaaaatgagtttttaaaaatgagatgaaaaataatttttgaaagttaaaattgtatttggacatgcattttatttgaaaagaatttgaagttttgtaagttaaaattttcaaaaacttcaaaaagttatttttgagatttgaagattttattttcaaaatttgcattataatctataaacaaatagatactatttgagaacaaaatttaaaaaataaagctttcaaacttatgacgaaagggaagcttaggataaaaaggggggaaatggcctgggagatgggtgggcaggttgggctgaagagaaatagacaacagtgcattaacatgtcaaatcatctttatccctctttaaaaacattattaggagtacttctttttttcttggggtgcaaaagcctaatacaagttaaaacacatattctctagctgctaagctataactttaactcattggtaccacgacgagtaggagaataaactttttgggcttttcttttcttttctttggttcccattttttgaactatcaatattttagtccaaacacacctgactctacagtgatctgatggccactataaatattggctttttgcagctccaaaatacaaatcggtcgaactcttcatatatattactcttaactttaaataaatagatttcttatatatgggttcaaaaatgtctgatccccttgtgattggtagagtgataggggaagttgttgattatttcactccaagtgttaagatgtctgttacttataacagcagcaagcatgtctataatggacatgaactctttccttcctcagtcacctctaaacctagggttgaagttcatggaggtgatttgagatctttctttacactggtacatactccttcgattttcactacttttaatttattaggggcgaagctagagttctagctacgggttcgttgtattaattgtgttaagaagtccacttaagctgtcttttttagaatttagaatccataaactcaaaatagtgactttgcttctaaattaatttttatgcatttctcttatatcgtgtatgtgaatattgaccccttattttttcttttttaccttaattgacagatcatgatagacccagatgttcctggtcctagtgatccatatctcagggaacatctacactggtaaagacatacgttttttaattactaactcattcaattttatcgccccttcttttccttgtttacttggagggaaaataatacgatctcgtcaagaagatcaaaaatcttcaggcttgttatttaggaacttgttcaaaaataccgttttgaaaagaacatatgagtttgttattaggtatttgactaaataggaacgatcatatggtgttcggacaagaaaatttttgtgaaaaggtccgcatactttaaaaaaaaaaaaaaaaaaaaaaaatccgccttgactcttgagtttctgcttcttggaaaaaacatttcttctttttttttttgggttttttgacctttatatattaattaaagacaccactgagacacttaattaaaaaattgtatatgggaacgcaaaaagaaaaaaaaacatgtgttattaatcttatgtcaatgccatcagcaactcaggaaaatacggtcgatatactgtgatttgcttgcgaaaggagcaaagaagaaatcttttgataatgtttgttatgacgatgcacttaacctaaaataagttaggggccgtttggtaaatgaaataaggataataatctcggaacaaagtttaggattaactttatcccatatttgatttggagtattagttaattgcgggataactttcaaattaaaatagtaggattagttatctcatatataaagtaaaatacctaatcccaataatataataggagacaactctaatttgcgtagacataatgtccagtctcactttgtatatttgtcatgacgcatattaagcatgaatgataatatttcgacaatcttgtggcatttgattacactcagcaaattataaatatgtccaataattgcattaataattacttgttcctcttatcattatagtgcctcattcactaaaccgaacccaaaagaacactgcaaaatggtcatatcatgtagtaacagaaaaaaaaaacgtactcgattttatgataaaatcaaagtgacatatgtgtcgctttgataattgacaaatacctgaaaaaagaatttgaccatctttacaggattgtcacagacattccaggcactacagattgctcgtttggtatgtatctttaacccaaagttcaagctatgaaatagtaacagcttttctttttaatattttatttgtcttaaatacatattttccttattataaatttattcgcctagtggtaacgggatcaggtattgattcgtatttaatttttattgttcaacaaaaaagagtacaaaaagaaagaattgattttctacacttagatttatatgcaatatctagaaatcagaagatcagcaatgagtttactaattcatcgatgtgtatatcgcacaatcaaatccaattactaataatactgatctaaaaatttcgatcagggagagaaatagttgggtatgaaatgccaaggccaaatattggaatccacaggtttgtatttctgctgttcaagcagaagaagaggcaaacattattgagtgcacctctctccagggatcgatttaatacgcgcaaattctcagaagaaaatgagcttgggtctcctgttgcagcagctttcttcaattgccagagggaaaccgctgccagaaggcgttga

SEQ ID NO: 11 - DNA, 2080 bp, Nicotiana tabacum
atgtctgttacttataacagcagcaagcatgtctataatggacatgaactctttccttcctcagtcacctctaaacctagggttgaagttcatggaggtgatttgagatctttctttacactggtacatactccttcgattttcactacttttaatttattaggggcgaagctagagttctagctacgggttcgttgtattaattgtgttaagaagtccacttaagctgtcttttttagaatttagaatccataaactcaaaatagtgactttgcttctaaattaatttttatgcatttctcttatatcgtgtatgtgaatattgaccccttattttttcttttttaccttaattgacagatcatgatagacccagatgttcctggtcctagtgatccatatctcagggaacatctacactggtaaagacatacgttttttaattactaactcattcaattttatcgccccttcttttccttgtttacttggagggaaaataatacgatctcgtcaagaagatcaaaaatcttcaggcttgttatttaggaacttgttcaaaaataccgttttgaaaagaacatatgagtttgttattaggtatttgactaaataggaacgatcatatggtgttcggacaagaaaatttttgtgaaaaggtccgcatactttaaaaaaaaaaaaaaaaaaaaaaaatccgccttgactcttgagtttctgcttcttggaaaaaacatttcttctttttttttttgggttttttgacctttatatattaattaaagacaccactgagacacttaattaaaaaattgtatatgggaacgcaaaaagaaaaaaaaacatgtgttattaatcttatgtcaatgccatcagcaactcaggaaaatacggtcgatatactgtgatttgcttgcgaaaggagcaaagaagaaatcttttgataatgtttgttatgacgatgcacttaacctaaaataagttaggggccgtttggtaaatgaaataaggataataatctcggaacaaagtttaggattaactttatcccatatttgatttggagtattagttaattgcgggataactttcaaattaaaatagtaggattagttatctcatatataaagtaaaatacctaatcccaataatataataggagacaactctaatttgcgtagacataatgtccagtctcactttgtatatttgtcatgacgcatattaagcatgaatgataatatttcgacaatcttgtggcatttgattacactcagcaaattataaatatgtccaataattgcattaataattacttgttcctcttatcattatagtgcctcattcactaaaccgaacccaaaagaacactgcaaaatggtcatatcatgtagtaacagaaaaaaaaaacgtactcgattttatgataaaatcaaagtgacatatgtgtcgctttgataattgacaaatacctgaaaaaagaatttgaccatctttacaggattgtcacagacattccaggcactacagattgctcgtttggtatgtatctttaacccaaagttcaagctatgaaatagtaacagcttttctttttaatattttatttgtcttaaatacatattttccttattataaatttattcgcctagtggtaacgggatcaggtattgattcgtatttaatttttattgttcaacaaaaaagagtacaaaaagaaagaattgattttctacacttagatttatatgcaatatctagaaatcagaagatcagcaatgagtttactaattcatcgatgtgtatatcgcacaatcaaatccaattactaataatactgatctaaaaatttcgatcagggagagaaatagttgggtatgaaatgccaaggccaaatattggaatccacaggtttgtatttctgctgttcaagcagaagaagaggcaaacattattgagtgcacctctctccagggatcgatttaatacgcgcaaattctcagaagaaaatgagcttgggtctcctgttgcagcagctttcttcaattgccagagggaaaccgctgccagaaggcgttga

SEQ ID NO: 12 - protein, 148 aa, Nicotiana tabacum
MSVTYNSSKHVYNGHELFPSSVTSKPRVEVHGGDLRSFFTLIMIDPDVPGPSDPYLREHLHWIVTDIPGTTDCSFGREIVGYEMPRPNIGIHRFVFLLFKQKKRQTLLSAPLSRDRFNTRKFSEENELGSPVAAAFFNCQRETAARRR

SEQ ID NO: 13 - DNA, 5167 bp, Nicotiana tabacum
tgaagttgtgtttggacatgcgttgtatttgagaaaaaattgaagttttgtgagaggaatttttttgaccccaaaactacataatttgaattattatttaaaaaaaatgatcatattacatgaacaaacagtgttttcaatttatttttgaaaaaaacagccaaaatctagccaaatgggagctaagtgtatgatcaagattcatgtcccaaatggaaaagaatattaacaaaaaaaagggcagtaaagaagaggtggctacaataggatcgcgcaaaagaaagatggaaaaaagaggaacaggaggggggaataagcagcacaagaagttattataagtcagctcttccagaaaggaatatggagaaaagttaacctcaggtttctataaataggaatgtccaactttcatttactagtttaagctgcagaaattctctttttcttgacatgaccttttcaccatctttaatttggtgggctttgtggtggagtccctttataccataggctctcctagaggatccataacattagattggtaaggttctaagtggactcacgatatgaaatttgtgatcgaacctataactcgtctgagttactgaatttgtaataaaatatttatacatatttaataaattttctaatataaatacagaatctaaacaaaaactattgagttcatccgtaccgatacctaatactctagctccaaccctgattctaatataatgaaaataaaaccacatctaggaagttcatgacctgttcttaccttaaatgccaaaggccttaaacctttgatagcttgagaatagccaaacaagtatagattccatctactttaattttctttctgattaagatatattgcaactcctgtaaatgcgcaaggagtcagctggttcttcccccatttctatattttttagtatcactttcttttcttaattattccttcttacatttgaatctttttccatcagctagctgttttgatagtagtaaaaatgcgaaggctcttcttactaatatttcaatgaccaatgaatttagatggagaagcaagttctattaaacgttcatgctagaaaataacaagtataatatttcattttcattttatataacgctcttgtcttttcttgtctatttaaacaagaatcaatttaactctcttaatgacatgctctttagtcacagaaaaattataacaaattgaagacattagttattaatgttcttttcgcactaaaagttttttaaaaattttttatcttaaatgtttgtgactaatcaaatatcatcatataaaattaatctgggaatatgacatttttcaatataactaatatggtgcaaattgcatacactacgcaataaatttgtggttagggtcatatcattagcctgtcaaatcatctttatccctctttctctaaacgacttcttttctcccttttttttcgcccctcaaacaaagcaaatagactattctctagctgctaattagctaaacaatgactttaactcgttgtgcccagaggagaataacctttatctctcttctcttttctttgtttccatctttaatttagacttctttttttggttttttatcccatattcggtatttattggagttcgattaaattcaaatttataataggaagtctcacattgagagtacgatgactccatactcaggattcgaatttgagatctttagttaaagatgaaagaatatcattcaaccacaacttttgttggtcccatctttatatctatatgttcttactatattttaatccatttcccacttccaatgatttaaagaagctataggataggtgcatttggaccactataaatataggttttgcagttctatgctccatacaaatatccagcaagaaactaaactatatatttactgagttactactaatagttttcactcaatctatttccactctttctcctcttcattatattatatggctcaaatgacagatccccttgtgattagtagggtggttggagatgttgttgattatttctctccaagtgttaagatgtgtgttatttataaccccagtaagcatgtctataatgggcatgaactctttccatcccttgttacctctaaacctaaggttgaagttcatggaggtgacatgagatccttctttacactggtaattaattcacactacttcaatagttttcttgttcttatattttattatctatctatatatatataataaaggagcggcaaagccaccatataaatgacaaatgtaaacttttaggacaaaactccaaaaaagttggagttttaaaattattttatatataaaataaataaataaataaataaataaactatcaattcaaattggggagtagtttcttactaatatgatagctatatctatatctatatctatctatatatgtaaaacatttatatgatgccaagtggcataaccactgataagatttttaaatttgaatatgaatgaattttaaatgaagttctaacttcttaaaaataaaccctaatataggttactatttttagtaatgattgaaattattattaaaatattttgttgaaaacaacatagagataaaatttgattattaaatttatgtattacaacaataataattattgaaaatattgctaaaattttcatgaaaggattcacccataattattagtataatagaaaactaaaaaattattaagtctaaagttctagatctctatatttataaacgtataaactgttattttattttctgaaaaaagcaaaaatactgaagagaaaaatgataaaaatattttaaaatatgtaagtcatgtgcaaataataaagtgaacaaatgatgtagtagtatactgaataagatatgtttttttgtcataaaataagtatatgcataactcatctcaataatttgctgactccatctgagtcaaaatatcttctaaattcaagcgaagataattatctatcgcattatttttttatcattaatataaggcaagacgaatctatatctcatatgggactttttaaatagatacatctttataaatgaaccactttatgagttttatcacgaattacaagtaagaataacttgaagattgaaagaatttttggatttatttaattataatatatttttattcattttaaattaatttatattttcaaattatttgtagcaacctatataattatgatatttgagtattatcttataagttatttgatgattgtcgtttgatttaattattgaactattactacaggggacataagatgataattataattttgtagaaacatatgatctaatgtgctcaaataaattactatcatactttgatatgactaatattctttaataatttttgcgcatcgggcgggtactaatactagttcttaaaaaaagggtagcgcgatgcacaaagcattccgcattcacacaggatcctaggaattgggtcgcaccccacagtctaccctaatgcaaacattagcgactactttcacggctcgaactcgtcacttatagatcatacagagacaaatttactgttgctccaagttccctttcttattttattattcttataatttctattcttatattgttataaattatttttttctttttgatagatcatgactgaccctgatgttcctggtcctagcgatccatatcttagggagcacttacattggtatgtatcatactatcatcaactttgaaagcttaaaacactgtaaagttgatgattcacaccaaagattttaatcgtcgtcgtgttacttccatataaatcagtatcgagaagtatgtggccatcactccatcaacgacaccaaaatgaaataaagagtccctatatcaatacaatataaattaatcttaaacatgaagttgactttaaattggataaattgtttccactactaagcttagcgtataaattagtcctttgactttcaattttgtataataatgcgaagctttttttcttgtaaatgcaatttttgtccttgagggtttgcaacttcttttttaaggaaaaaaaaaagactaaagttgtgtgacactaaaaccaagagttagcttaatacttcatggacacacgttagcataaaacatataaccgatattcaaaattacaaaaatgatagaatcataatttttgtttctatttaaaaaggaagtaagccaaattactactaacatagtggacttaaagggtattaattttttgttattttaatgatatctgttcatgacttcttgactacttctactcctttatatcaatcaaattataatttacttcgtttgactatctaatttacagggtaattacagacattccaggcactacagattcctcgtttggtatggaataatattgtattccttttttacttttctgcctagcatttctaaatagagtagtccgatacacgaaatatttcactttacgcaggatccagaaataaaggaccataccccaattgggtgtaatataagtagtcatgggcgcatgcagtattttagtgacgggtttaattgcactcataattttggacgcttagcataaagtagtagatatgtatccataacttcaaaaatataataggttcaatgttaaaaatttcaaaagagatgaactcatagagtttaaatcatgatccgcctctgtaggcagtctaccctaatgaaagaatcagtggctgatttcacagttcaaaaccgtaacctatgaatcacataaagccaactttaccatcgctccaagactcgccttcttctgcctaacattactactgctaataaagagaattttaataaaactactaatgctaattattattctttgctaaaatcttcatcaggaaaagaagtggtgggctatgaaatgccaatgcctaacattggaatccataggtttgtgtttctgctcttcaagcagaagaagaggcaaacagtgagcgcaccattatccagggaccgattcaatacgcggaaatacgcagaagaaaatgagcttggctctccagttgctgctgttttcttcaactgccaaagggaaaccgcggccagaaagcgttga

SEQ ID NO: 14 - DNA, 3167 bp, Nicotiana tabacum
atggctcaaatgacagatccccttgtgattagtagggtggttggagatgttgttgattatttctctccaagtgttaagatgtgtgttatttataaccccagtaagcatgtctataatgggcatgaactctttccatcccttgttacctctaaacctaaggttgaagttcatggaggtgacatgagatccttctttacactggtaattaattcacactacttcaatagttttcttgttcttatattttattatctatctatatatatataataaaggagcggcaaagccaccatataaatgacaaatgtaaacttttaggacaaaactccaaaaaagttggagttttaaaattattttatatataaaataaataaataaataaataaataaactatcaattcaaattggggagtagtttcttactaatatgatagctatatctatatctatatctatctatatatgtaaaacatttatatgatgccaagtggcataaccactgataagatttttaaatttgaatatgaatgaattttaaatgaagttctaacttcttaaaaataaaccctaatataggttactatttttagtaatgattgaaattattattaaaatattttgttgaaaacaacatagagataaaatttgattattaaatttatgtattacaacaataataattattgaaaatattgctaaaattttcatgaaaggattcacccataattattagtataatagaaaactaaaaaattattaagtctaaagttctagatctctatatttataaacgtataaactgttattttattttctgaaaaaagcaaaaatactgaagagaaaaatgataaaaatattttaaaatatgtaagtcatgtgcaaataataaagtgaacaaatgatgtagtagtatactgaataagatatgtttttttgtcataaaataagtatatgcataactcatctcaataatttgctgactccatctgagtcaaaatatcttctaaattcaagcgaagataattatctatcgcattatttttttatcattaatataaggcaagacgaatctatatctcatatgggactttttaaatagatacatctttataaatgaaccactttatgagttttatcacgaattacaagtaagaataacttgaagattgaaagaatttttggatttatttaattataatatatttttattcattttaaattaatttatattttcaaattatttgtagcaacctatataattatgatatttgagtattatcttataagttatttgatgattgtcgtttgatttaattattgaactattactacaggggacataagatgataattataattttgtagaaacatatgatctaatgtgctcaaataaattactatcatactttgatatgactaatattctttaataatttttgcgcatcgggcgggtactaatactagttcttaaaaaaagggtagcgcgatgcacaaagcattccgcattcacacaggatcctaggaattgggtcgcaccccacagtctaccctaatgcaaacattagcgactactttcacggctcgaactcgtcacttatagatcatacagagacaaatttactgttgctccaagttccctttcttattttattattcttataatttctattcttatattgttataaattatttttttctttttgatagatcatgactgaccctgatgttcctggtcctagcgatccatatcttagggagcacttacattggtatgtatcatactatcatcaactttgaaagcttaaaacactgtaaagttgatgattcacaccaaagattttaatcgtcgtcgtgttacttccatataaatcagtatcgagaagtatgtggccatcactccatcaacgacaccaaaatgaaataaagagtccctatatcaatacaatataaattaatcttaaacatgaagttgactttaaattggataaattgtttccactactaagcttagcgtataaattagtcctttgactttcaattttgtataataatgcgaagctttttttcttgtaaatgcaatttttgtccttgagggtttgcaacttcttttttaaggaaaaaaaaaagactaaagttgtgtgacactaaaaccaagagttagcttaatacttcatggacacacgttagcataaaacatataaccgatattcaaaattacaaaaatgatagaatcataatttttgtttctatttaaaaaggaagtaagccaaattactactaacatagtggacttaaagggtattaattttttgttattttaatgatatctgttcatgacttcttgactacttctactcctttatatcaatcaaattataatttacttcgtttgactatctaatttacagggtaattacagacattccaggcactacagattcctcgtttggtatggaataatattgtattccttttttacttttctgcctagcatttctaaatagagtagtccgatacacgaaatatttcactttacgcaggatccagaaataaaggaccataccccaattgggtgtaatataagtagtcatgggcgcatgcagtattttagtgacgggtttaattgcactcataattttggacgcttagcataaagtagtagatatgtatccataacttcaaaaatataataggttcaatgttaaaaatttcaaaagagatgaactcatagagtttaaatcatgatccgcctctgtaggcagtctaccctaatgaaagaatcagtggctgatttcacagttcaaaaccgtaacctatgaatcacataaagccaactttaccatcgctccaagactcgccttcttctgcctaacattactactgctaataaagagaattttaataaaactactaatgctaattattattctttgctaaaatcttcatcaggaaaagaagtggtgggctatgaaatgccaatgcctaacattggaatccataggtttgtgtttctgctcttcaagcagaagaagaggcaaacagtgagcgcaccattatccagggaccgattcaatacgcggaaatacgcagaagaaaatgagcttggctctccagttgctgctgttttcttcaactgccaaagggaaaccgcggccagaaagcgttga

SEQ ID NO: 15 - protein, 173 aa, Nicotiana tabacum
MAQMTDPLVISRVVGDVVDYFSPSVKMCVIYNPSKHVYNGHELFPSLVTSKPKVEVHGGDMRSFFTLIMTDPDVPGPSDPYLREHLHWVITDIPGTTDSSFGKEVVGYEMPMPNIGIHRFVFLLFKQKKRQTVSAPLSRDRFNTRKYAEENELGSPVAAVFFNCQRETAARKR

SEQ ID NO: 16 - DNA, 4569 bp, Nicotiana tabacum
  misc_feature (1896)..(1896): n is a, c, g, or t
ccttatgggttctcagcatttgggcaaaagtgatactttaagcaagtgaggaagttttttaatgttggccggaaagatgcctgtgggtgctgtttgggggaaaaaaacaaaagctcgggtaaattatcaatacccgagttggttcctttcgtttgccactggaccaactcctgattttgcttatatatgggttccaaactaaaaatacttatatatttaataaatttatcaatacaaatacaaggctcgggtaaaagttattaggttctcggaaacccatacccgatactatggatccgcccctgcttatccctaccttgtgtgaggtagaaacgcttttgataaggttatttaaaagtaaaagaataagtttaatgtgacaatttgaatggttgagacaacatgccaaaagctaatttaagggattttatttgacatttatatatgggagagaagaaaaagtattgcccagtatattattttaagctctacaaccaatcaagaatcaattcctagaatccattcaggtgtcaaagaatactgacatgatataataaaatacaatttatatcacatcagtatttgctttttcttgggagattagataaaaagagatcagaaatggagttttatggtactaggagaattcaaggatttactacttttgtggcacaacataagctcccaatttttttaaggaatttataaaagttggttttctaagtacttacaattgtcaaatttacaagtcatttagtacataaaaagaaacccaatgatgaggttcaggaaaaaaaaaaatcctatactgtgatttcctagttggcgttcggacataaaaattatgaaattccgaaaaaaaaaattgttttaagttgaaaatggtatgtgaaaattaaagttatatatggacataaatataatttggagctgtttttgaatttttgtgagtgctttgaagtgaaattttctaaaaacagctttttggagtttttcaaattccggagttcaacttcaagcgaaaaattaaaattttcatgatcaaatgttgattccgaaaaaagtgaaaaaattcgaaaaaaagatttttttttttatggccaaacagacctaactagtttcattttagtcattaagggtagaattgaaagaattttaaattaaagtatttttagatatataaaaataatgtactttttaaaacacacaaaaaaaggagtgccatatattaatttaatataaggatatatagtggatgcattcataactaacattaaccaaaagcatttattgatcctattttgacaccattttattttaatacaattcataaatttcaagaatttgaatacattagcttaatctcacttaaattttgaggtgatgcctgttctctttctagtcacaactttaatgtacattttatatgtcaaattaatacctgaatttgtaacccatcaaatatcgccacataatatgaaacagtgaaaatatcttatattcctgtattttatgactaagacattaagtagctaacaacgatcgaaaaacattcctaataacaagcgaattacaactctgtcggataatcgtctgaaaccctaaaaagctactgaaatgatttcctactagtataattccgatgaaattttgttcgaaaattctataagaaatacacgtatttttagtagtgaaaaaagatttgttgtaatttttttaggtggggtggggtgatttggggagggttggggagtaggacctcaaaaacaaagaattttaatactttggagtttccttaggtcccatgttttatactttcttttattctccttcaccattatagctataacttagtacatatatatatatatatatatatatatatatatatatatnatataaggtgtccatctgatcaagtatccaatacaaaccattcttaagtctttgaaaatttctctttttttccttatctctatctctgtctaattttctttattatggcaagaagtttagagcctctaattgttgggagagtagtaggagatgttcttgattcatttagtcctataatgaaaatgacaatatcatataacaacaaattagtgtgcaatggccatgaactccttccttctgttgtcactgctagacctaaagttgaagttcaagggggagatttgagaactttcttcacattggtatttttttcttgatttctacttaatttccaagatcatcaagttcccattatttctttaaaaaaaaaaaaagcagttcggtgcactaaactcccgctatgcgcggggttcggtgaagcaccgaaccataagggtctattgtacgcaaccttaccctgcatttatgcaagaggcttgctcaccattacaagttatattaatttaacatgttatatataaccacaaaggctgtcgtgggatggtaaatatccttctatccttaatcagaagtttcgggttcaagttatagccctaggaatatagtcgtctttggtagggatcctttacccccaaaactttccgccgtgaatccagattagtaaacctcaaagcgggtatcgggcattggatgacaaaccaaaaaaacttcaacgtgttatagcatgttataacttattacagttaatttagttttccagtcgatactatattaaatagagtgcctgtaatttactttggagtgatttgattgttattttttcgcatcgtcagtacataaaacttatattaattttcgaatatgtaggtcatgacagaccctgatgttcctggccctagtgatccttatctaagagagcatctccactggtatgccctaaactcaatttttttttaaaaaaaaaaaatagaaaatgagaaaaaatatgtaaaaatctacaaatatgagaagatcatgattaattggaactatttttactgactatttgacaggatagtaactgacattccaggtaccactgatgctacttttggtaagttctctgtatcttctgcaaaattacaagcacatgtgaagataaaagaagtttttctattattcacttattttgtctagctagttatatagaataattataagatcaacaattttgtatagtagtgaatgttggacttctaaagtcgaacatgtccacttgatgagtgtcacaaaaatgtagaaactaaacaatcgtttggacataaaaaaaaaagtaagtttttttgagttaaattgaaaaagaaaatatttagaatttgaaattgtggatatacatttaaattgaaaagcattgcagttttgtaaggaaaataaactttcatatacataaaaaagtgattttttggaaactcatcttcaagaatatttttaaaaatttccgtccaatgtataaccaaacattattttgaaaaagattaaaaaaaggaaaaactttaggaacaacgggtcccaagataaatgtgtctagtcatataagattagataaattaggattttattatatttggtagaaggtgcaagaagcatatgtaaataataaattgagaagtcacttaagatattttgatcatgtcccacatcgataacaagaggtaccattctatatatgttaaatcatggtaagttaaagtattatatcacatattaaatggtgatataatagacctaaatcacatgaaacgaaattgtcccgaaaggtctataaatttttgaaattcatgtagacgaagctaaaagtaggatacaataaaaaaaaaattaaagatctatattggcgatactatttagttgggattgcattttagttattctagtacatttactttaatctaatttttgctagctaggagtcttttaatcttattagaaatttacataccaaaaaatttagagaacttgctaggacaattggtatttctttatataatattgtggaagttgtattagagtatgttgtttacattacactctttgagtgcgttccttctccgaactagctaatgcatgaacacgagatgccttctgcaccgtgctaccctattaatatataaaaaaatggtagcccggtgcattaagctcccgctatgcgcgggttccgaaaaaggatcagaccacaagggtctatgtttgcaaccttacttgtatttctgcaagaaactgtttccacggctcgaacccatgatcttctggtcacatgacaataactttaccggttacaccaaggttccccttcacgcgctgcccttttaatattgtctattaatatttcctactagagttatacacccctttgttattactcactcttagggtgattattaacatataatatgtttaatatttatactaaaaacaggacgagaattggttagctatgagattccaatgccaaatattggaatccataggtttgtatttgtacttttcaagcaaaaacgaagacaatcagttagctctcctacttcaagggatcacttcaacactagaaattttgctgaagaaaatgatcttggccaacctgttgctgctgttttcttcaatgcacagcgagaaaccgccgcacgaagacgctaa

SEQ ID NO: 17 - DNA, 2569 bp, Nicotiana tabacum
atggcaagaagtttagagcctctaattgttgggagagtagtaggagatgttcttgattcatttagtcctataatgaaaatgacaatatcatataacaacaaattagtgtgcaatggccatgaactccttccttctgttgtcactgctagacctaaagttgaagttcaagggggagatttgagaactttcttcacattggtatttttttcttgatttctacttaatttccaagatcatcaagttcccattatttctttaaaaaaaaaaaaagcagttcggtgcactaaactcccgctatgcgcggggttcggtgaagcaccgaaccataagggtctattgtacgcaaccttaccctgcatttatgcaagaggcttgctcaccattacaagttatattaatttaacatgttatatataaccacaaaggctgtcgtgggatggtaaatatccttctatccttaatcagaagtttcgggttcaagttatagccctaggaatatagtcgtctttggtagggatcctttacccccaaaactttccgccgtgaatccagattagtaaacctcaaagcgggtatcgggcattggatgacaaaccaaaaaaacttcaacgtgttatagcatgttataacttattacagttaatttagttttccagtcgatactatattaaatagagtgcctgtaatttactttggagtgatttgattgttattttttcgcatcgtcagtacataaaacttatattaattttcgaatatgtaggtcatgacagaccctgatgttcctggccctagtgatccttatctaagagagcatctccactggtatgccctaaactcaatttttttttaaaaaaaaaaaatagaaaatgagaaaaaatatgtaaaaatctacaaatatgagaagatcatgattaattggaactatttttactgactatttgacaggatagtaactgacattccaggtaccactgatgctacttttggtaagttctctgtatcttctgcaaaattacaagcacatgtgaagataaaagaagtttttctattattcacttattttgtctagctagttatatagaataattataagatcaacaattttgtatagtagtgaatgttggacttctaaagtcgaacatgtccacttgatgagtgtcacaaaaatgtagaaactaaacaatcgtttggacataaaaaaaaaagtaagtttttttgagttaaattgaaaaagaaaatatttagaatttgaaattgtggatatacatttaaattgaaaagcattgcagttttgtaaggaaaataaactttcatatacataaaaaagtgattttttggaaactcatcttcaagaatatttttaaaaatttccgtccaatgtataaccaaacattattttgaaaaagattaaaaaaaggaaaaactttaggaacaacgggtcccaagataaatgtgtctagtcatataagattagataaattaggattttattatatttggtagaaggtgcaagaagcatatgtaaataataaattgagaagtcacttaagatattttgatcatgtcccacatcgataacaagaggtaccattctatatatgttaaatcatggtaagttaaagtattatatcacatattaaatggtgatataatagacctaaatcacatgaaacgaaattgtcccgaaaggtctataaatttttgaaattcatgtagacgaagctaaaagtaggatacaataaaaaaaaaattaaagatctatattggcgatactatttagttgggattgcattttagttattctagtacatttactttaatctaatttttgctagctaggagtcttttaatcttattagaaatttacataccaaaaaatttagagaacttgctaggacaattggtatttctttatataatattgtggaagttgtattagagtatgttgtttacattacactctttgagtgcgttccttctccgaactagctaatgcatgaacacgagatgccttctgcaccgtgctaccctattaatatataaaaaaatggtagcccggtgcattaagctcccgctatgcgcgggttccgaaaaaggatcagaccacaagggtctatgtttgcaaccttacttgtatttctgcaagaaactgtttccacggctcgaacccatgatcttctggtcacatgacaataactttaccggttacaccaaggttccccttcacgcgctgcccttttaatattgtctattaatatttcctactagagttatacacccctttgttattactcactcttagggtgattattaacatataatatgtttaatatttatactaaaaacaggacgagaattggttagctatgagattccaatgccaaatattggaatccataggtttgtatttgtacttttcaagcaaaaacgaagacaatcagttagctctcctacttcaagggatcacttcaacactagaaattttgctgaagaaaatgatcttggccaacctgttgctgctgttttcttcaatgcacagcgagaaaccgccgcacgaagacgctaa

SEQ ID NO: 18 - protein, 172 aa, Nicotiana tabacum
MARSLEPLIVGRVVGDVLDSFSPIMKMTISYNNKLVCNGHELLPSVVTARPKVEVQGGDLRTFFTLVMTDPDVPGPSDPYLREHLHWIVTDIPGTTDATFGRELVSYEIPMPNIGIHRFVFVLFKQKRRQSVSSPTSRDHFNTRNFAEENDLGQPVAAVFFNAQRETAARRR

SEQ ID NO: 19 - DNA, 4652 bp, Nicotiana tabacum
atccccagaggcggatctaggatttgaaccttatgggttctcagcatttgggcaaaagtgatactttaagcaagtgaggaagttttttaatgttggccggaaagatgcctgtgggtgctgtttgggggaaaaaaacaaaagctcgggtaaattatcaatacccgagttggttcctttcgtttgccactggaccaactcctgattttgcttatatatgggttccaaactaaaaatacttatatatttaataaatttatcaatacaaatacaaggctcgggtaaaagttattaggttctcggaaacccatacccgatactatggatccgcccctgcttatccctaccttgtgtgaggtagaaacgcttttgataaggttatttaaaagtaaaagaataagtttaatgtgacaatttgaatggttgagacaacatgccaaaagctaatttaagggattttatttgacatttatatatgggagagaagaaaaagtattgcccagtatattattttaagctctacaaccaatcaagaatcaattcctagaatccattcaggtgtcaaagaatactgacatgatataataaaatacaatttatatcacatcagtatttgctttttcttgggagattagataaaaagagatcagaaatggagttttatggtactaggagaattcaaggatttactacttttgtggcacaacataagctcccaatttttttaaggaatttataaaagttggttttctaagtacttacaattgtcaaatttacaagtcatttagtacataaaaagaaacccaatgatgaggttcaggaaaaaaaaaaaatcctatactgtgatttcctagttggcgttcggacataaaaattatgaaattccgaaaaaaaaaattgttttaagttgaaaatggtatgtgaaaattaaagttatatatggacataaatataatttggagctgtttttgaatttttgtgagtgctttgaagtgaaattttctaaaaacagctttttggagtttttcaaattccggagttcaacttcaagcgaaaaattaaaattttcatgatcaaatgttgattccgaaaaaagtgaaaaaattcgaaaaaaagatttttttttttatggccaaacagacctaactagtttcattttagtcattaagggtagaattgaaagaattttaaattaaagtatttttagatatataaaaataatgtactttttaaaacacacaaaaaaaggagtgccatatattaatttaatataaggatatatagtggatgcattcataactaacattaaccaaaagcatttattgatcctattttgacaccattttattttaatacaattcataaatttcaagaatttgaatacattagcttaatctcacttaaattttgaggtgatgcctgttctctttctagtcacaactttaatgtacattttatatgtcaaattaatacctgaatttgtaacccatcaaatatcgccacataatatgaaacagtgaaaatatcttatattcctgtattttatgactaagacattaagtagctaacaacgatcgaaaaacattcctaataacaagcgaattacaactctgtcggataatcgtctgaaaccctaaaaagctactgaaatgatttcctactagtataattccgatgaaattttgttcgaaaattctataagaaatacacgtatttttagtagtgaaaaaagatttgttgtaatttttttaggtggggtggggtgatttggggagggttggggagtaggacctcaaaaacaaagaattttaatactttggagtttccttaggtcccatgttttatactttcttttattctccttcaccattatagctataacttagtacatatatatatatggtggccctctgatccaatgtaaaatgcaaaccattcttaagatctttgaaatttctctcttttttttctttatctctatctctgtctaattctctctattatggcaagaagtttggagcctctaatagttgggagagtagtaggagatgttcttgattcatttagtcctatagtgaaaatgacaattacttataacaacaaattagtgtgcaatggtcatgaattctttccttctattgtcacttctagacctaaggttgaagttcaaggaggagatttgagaactttcttcacactggtaatttttcttgattttttccttaattccaagatcatcaagttccatttatttctttacaagttatattaatttaaccctttataatcaccaaaggctggcgtgggttgctaagtaaccttccatcgttaatcagatgtttcgggttcgagctagccctgggattacaatcgttttttgtaggaagcgctttaacccccaaaatttttcagcacgaacccggattagtaaacctcaaaactcgtgccaaatactagatgacaaaccaaaagagttttcaacctgttataacatatgttacttgttacaattattagttttccggtcaatagtatattatgtaattttctttgaagtgacttgattgttattttttcacattatcagtgcataaaacttatactattattttttaatatgtaggtcatgacagaccctgatgttcccggccctagtgatccttatctacgagagcatctccactggtacactctctataatagtttcatttgttccgaattttcttggctgttatataaaaaatatattataacatagcatgaaaattggttccacaaaaacttaatttttatagtgaataattgttatatattgatattgttatagagaggtctgtctatatgccctaaactcaatgaaaaaaaatagaaaatgagaaaaaatatgtaaaatctacaaatatgagaagatcatttttagttgaaactatccttatatactactgaatatttagctggcaaataaaattgacagtgttttactgattgtttgacaggatagtaactgacattccaggtaccactgatgctacttttggtaagttttattagtttcttctgcaagattacaagcacatgtgaagaagatacaagatgtttttccattactcacttattttgtcttgctaataattatatagaacaattgtaagatcaacagtgttatataatagtgaatgttggacttctaaagtcgaacatgtccacatgatgagcgtcacaaaaatgcagatacgagctcgtttggattgacttaaaaaatgtggtttttcagcaaaaataacttttaagccaaaaaacaataagttagggttgtccacctttttgcttttggcttaatttaagcattttaaaatttattttaagcaatttttgacttagccaaacaccgaaaaaagctaaaagaaacttaaaagctgatttgactagcttaaaagtaaatccaaacaccctctaactaagcatttggacataaaaaaaatatgtcatttttgaaaaaagtagttcttttgagttaagtcaaaaaagaatatataaaatttgaaattgtatttagacatgcatttcacttgaaaattattagagttttatgagaaaaatgaacttttagatgaaaaagtggtttttggaaactcatcttcaagaatttttccaaaacttcagtccaatcgtataaccaaacattattttgataaaaacatcgaaaataaaaataaatctatggagaaacgggtcccaagataaatgtgtctagtcatataagattattcaaaattaagaatttatcacatttgtaaaagatgtaagtagcatatgtaaatgataaaatgagaagtcacttgagatgttttgatcatgtcctacgtcgatcttcagaggtaccattccgtatacgtgattggtaagtaaaggtattaaaaagagacataatggacctaaattacgtgaaacgaaattgtcttgaaaagtctttcaaatttttgaaatccatgtagacgaatcgaaaagtagggcacaatgaaatatgatcaaaggtttataatggtgatacaagttagttgggattacgttttagttatgccagtatatttactttaatctaatattttcttggagttttttaatcttattagaaatttacttaccaaaaatttagagaacttgctagaacaatataattgataattcttcatatatattgtcttcgagctgtagaaacagccactaatgtttgcattaggatatgttgtctacatcacacttattgtgtgttgccctcaccggaccctgcatgaacgtatgatgccttatgcaccgcgccccttttaatattatttattaattaatatttcctgctagagttatactcctttgttattactcattcttaggttgatgattaacttataatatgcttaatctttatactaaaaataggaagagaattggttagctatgagattccaaggccaaatattggaatccataggtttgtatttgtacttttcaagcaaagacgaagacaatcagttagccctcctacttcaagggaaaacttcaacactagaaattttgccgaagaaaatgatcttagccaacctgttgctgctgttttcttcaatgcacagcgagaaaccgccgcgcgaagacgctaa

SEQ ID NO: 20 - DNA, 2653 bp, Nicotiana tabacum
atggcaagaagtttggagcctctaatagttgggagagtagtaggagatgttcttgattcatttagtcctatagtgaaaatgacaattacttataacaacaaattagtgtgcaatggtcatgaattctttccttctattgtcacttctagacctaaggttgaagttcaaggaggagatttgagaactttcttcacactggtaatttttcttgattttttccttaattccaagatcatcaagttccatttatttctttacaagttatattaatttaaccctttataatcaccaaaggctggcgtgggttgctaagtaaccttccatcgttaatcagatgtttcgggttcgagctagccctgggattacaatcgttttttgtaggaagcgctttaacccccaaaatttttcagcacgaacccggattagtaaacctcaaaactcgtgccaaatactagatgacaaaccaaaagagttttcaacctgttataacatatgttacttgttacaattattagttttccggtcaatagtatattatgtaattttctttgaagtgacttgattgttattttttcacattatcagtgcataaaacttatactattattttttaatatgtaggtcatgacagaccctgatgttcccggccctagtgatccttatctacgagagcatctccactggtacactctctataatagtttcatttgttccgaattttcttggctgttatataaaaaatatattataacatagcatgaaaattggttccacaaaaacttaatttttatagtgaataattgttatatattgatattgttatagagaggtctgtctatatgccctaaactcaatgaaaaaaaatagaaaatgagaaaaaatatgtaaaatctacaaatatgagaagatcatttttagttgaaactatccttatatactactgaatatttagctggcaaataaaattgacagtgttttactgattgtttgacaggatagtaactgacattccaggtaccactgatgctacttttggtaagttttattagtttcttctgcaagattacaagcacatgtgaagaagatacaagatgtttttccattactcacttattttgtcttgctaataattatatagaacaattgtaagatcaacagtgttatataatagtgaatgttggacttctaaagtcgaacatgtccacatgatgagcgtcacaaaaatgcagatacgagctcgtttggattgacttaaaaaatgtggtttttcagcaaaaataacttttaagccaaaaaacaataagttagggttgtccacctttttgcttttggcttaatttaagcattttaaaatttattttaagcaatttttgacttagccaaacaccgaaaaaagctaaaagaaacttaaaagctgatttgactagcttaaaagtaaatccaaacaccctctaactaagcatttggacataaaaaaaatatgtcatttttgaaaaaagtagttcttttgagttaagtcaaaaaagaatatataaaatttgaaattgtatttagacatgcatttcacttgaaaattattagagttttatgagaaaaatgaacttttagatgaaaaagtggtttttggaaactcatcttcaagaatttttccaaaacttcagtccaatcgtataaccaaacattattttgataaaaacatcgaaaataaaaataaatctatggagaaacgggtcccaagataaatgtgtctagtcatataagattattcaaaattaagaatttatcacatttgtaaaagatgtaagtagcatatgtaaatgataaaatgagaagtcacttgagatgttttgatcatgtcctacgtcgatcttcagaggtaccattccgtatacgtgattggtaagtaaaggtattaaaaagagacataatggacctaaattacgtgaaacgaaattgtcttgaaaagtctttcaaatttttgaaatccatgtagacgaatcgaaaagtagggcacaatgaaatatgatcaaaggtttataatggtgatacaagttagttgggattacgttttagttatgccagtatatttactttaatctaatattttcttggagttttttaatcttattagaaatttacttaccaaaaatttagagaacttgctagaacaatataattgataattcttcatatatattgtcttcgagctgtagaaacagccactaatgtttgcattaggatatgttgtctacatcacacttattgtgtgttgccctcaccggaccctgcatgaacgtatgatgccttatgcaccgcgccccttttaatattatttattaattaatatttcctgctagagttatactcctttgttattactcattcttaggttgatgattaacttataatatgcttaatctttatactaaaaataggaagagaattggttagctatgagattccaaggccaaatattggaatccataggtttgtatttgtacttttcaagcaaagacgaagacaatcagttagccctcctacttcaagggaaaacttcaacactagaaattttgccgaagaaaatgatcttagccaacctgttgctgctgttttcttcaatgcacagcgagaaaccgccgcgcgaagacgctaa

SEQ ID NO: 21 - protein, 172 aa, Nicotiana tabacum
MARSLEPLIVGRVVGDVLDSFSPIVKMTITYNNKLVCNGHEFFPSIVTSRPKVEVQGGDLRTFFTLVMTDPDVPGPSDPYLREHLHWIVTDIPGTTDATFGRELVSYEIPRPNIGIHRFVFVLFKQRRRQSVSPPTSRENFNTRNFAEENDLSQPVAAVFFNAQRETAARRR

SEQ ID NO: 22 - DNA, 58 bp, Nicotiana tabacum
agttaaaatgacagtcacttacaacaataaacaagtttgcaatggccaagagctcttc

SEQ ID NO: 23 - DNA, 58 bp, Nicotiana tabacum
gaagagctcttggccattgcaaacttgtttattgttgtaagtgactgtcattttaact

SEQ ID NO: 24 - DNA, 482 bp, Nicotiana tabacum
ggtaccacaagtttgtacaaaaaagcaggctaagcttgtcgaccatggagttaaaatgacagtcacttacaacaataaacaagtttgcaatggccaagagctcttctggtaacctttaatgtttaaccgttcacatttctaatatttacttatttgtaacatgtcgtcacgtgttagtttcattctttttatgaaccaaacatgcatgcaaagatatttttagatatttggacggcgagtgagatttgaaactaggaccgtttgcctgatacaatattaaaatatgtaaccattttatgtacaagtttaaactgttgatagtagcatattttttacttttatttaagtatactatattccaacaggtaagttaacgaagagctcttggccattgcaaacttgtttattgttgtaagtgactgtcattttaactggcgcgcccgggcaattgacccagctttcttgtacaaagtggtgagctc

SEQ ID NO: 25 - DNA, 88 bp, Nicotiana tabacum
tgcagtcactattagacctagggttgaagttcaaggtggtgatatgagaactttcttcacattggtcatcacagatcctgatgtacct

SEQ ID NO: 26 - DNA, 88 bp, Nicotiana tabacum
aggtacatcaggatctgtgatgaccaatgtgaagaaagttctcatatcaccaccttgaacttcaaccctaggtctaatagtgactgca

SEQ ID NO: 27 - DNA, 88 bp, Nicotiana tabacum
tgcggtcaccattagacctagggttgaggttcaaggtggtgatatgagaactttcttcacattggtcatgacagaccctgatgttcct

SEQ ID NO: 28 - DNA, 88 bp, Nicotiana tabacum
aggaacatcagggtctgtcatgaccaatgtgaagaaagttctcatatcaccaccttgaacctcaaccctaggtctaatggtgaccgca

SEQ ID NO: 29 - DNA, 78 bp, Nicotiana tabacum
catgaactctttccttcctcagtcacctctaaacctagggttgaagttcatggaggtgatttgagatctttctttaca

SEQ ID NO: 30 - DNA, 78 bp, Nicotiana tabacum
tgtaaagaaagatctcaaatcacctccatgaacttcaaccctaggtttagaggtgactgaggaaggaaagagttcatg

SEQ ID NO: 31 - DNA, 522 bp, Nicotiana tabacum
ggtaccacaagtttgtacaaaaaagcaggctaagcttgtcgaccatggcatgaactctttccttcctcagtcacctctaaacctagggttgaagttcatggaggtgatttgagatctttctttacatggtaacctttaatgtttaaccgttcacatttctaatatttacttatttgtaacatgtcgtcacgtgttagtttcattctttttatgaaccaaacatgcatgcaaagatatttttagatatttggacggcgagtgagatttgaaactaggaccgtttgcctgatacaatattaaaatatgtaaccattttatgtacaagtttaaactgttgatagtagcatattttttacttttatttaagtatactatattccaacaggtaagttaactgtaaagaaagatctcaaatcacctccatgaacttcaaccctaggtttagaggtgactgaggaaggaaagagttcatgggcgcgcccgggcaattgacccagctttcttgtacaaagtggtgagctc

SEQ ID NO: 32 - DNA, 121 bp, Nicotiana tabacum
gaaagaaatagttggctatgaaatgccaaggccaaatattggaattcacaggtttgtatttctgctgttcaagcagaagaagaggcaaacagtattgactgcacctctctccagggatcga

SEQ ID NO: 33 - DNA, 121 bp, Nicotiana tabacum
tcgatccctggagagaggtgcagtcaatactgtttgcctcttcttctgcttgaacagcagaaatacaaacctgtgaattccaatatttggccttggcatttcatagccaactatttctttc

SEQ ID NO: 34 - DNA, 110 bp, Nicotiana tabacum
gagagaaatagttgggtatgaaatgccaaggccaaatattggaatccacagcagctttcttcaattgccagagggaaaccgctgccagaaggcgttgaagaagatgttta

SEQ ID NO: 35 - DNA, 110 bp, Nicotiana tabacum
taaacatcttcttcaacgccttctggcagcggtttccctctggcaattgaagaaagctgctgtggattccaatatttggccttggcatttcatacccaactatttctctc

SEQ ID NO: 36 - DNA, 138 bp, Nicotiana tabacum
atggctcaaatgacagatccccttgtgattagtagggtggttggagatgttgttgattatttctctccaagtgttaagatgtgtgttatttataaccccagtaagcatgtctataatgggcatgaactctttccatcc

SEQ ID NO: 37 - DNA, 138 bp, Nicotiana tabacum
ggatggaaagagttcatgcccattatagacatgcttactggggttataaataacacacatcttaacacttggagagaaataatcaacaacatctccaaccaccctactaatcacaaggggatctgtcatttgagccat

SEQ ID NO: 38 - DNA, 642 bp, Nicotiana tabacum
ggtaccacaagtttgtacaaaaaagcaggctaagcttgtcgaccatggatggctcaaatgacagatccccttgtgattagtagggtggttggagatgttgttgattatttctctccaagtgttaagatgtgtgttatttataaccccagtaagcatgtctataatgggcatgaactctttccatcctggtaacctttaatgtttaaccgttcacatttctaatatttacttatttgtaacatgtcgtcacgtgttagtttcattctttttatgaaccaaacatgcatgcaaagatatttttagatatttggacggcgagtgagatttgaaactaggaccgtttgcctgatacaatattaaaatatgtaaccattttatgtacaagtttaaactgttgatagtagcatattttttacttttatttaagtatactatattccaacaggtaagttaacggatggaaagagttcatgcccattatagacatgcttactggggttataaataacacacatcttaacacttggagagaaataatcaacaacatctccaaccaccctactaatcacaaggggatctgtcatttgagccatggcgcgcccgggcaattgacccagctttcttgtacaaagtggtgagctc

SEQ ID NO: 39 - DNA, 93 bp, Nicotiana tabacum
tagtcctatagtgaaaatgacaattacttataacaacaaattagtgtgcaatggtcatgaattctttccttctattgtcacttctagacctaa

SEQ ID NO: 40 - DNA, 93 bp, Nicotiana tabacum
ttaggtctagaagtgacaatagaaggaaagaattcatgaccattgcacactaatttgttgttataagtaattgtcattttcactataggacta

SEQ ID NO: 41 - DNA, 552 bp, Nicotiana tabacum
ggtaccacaagtttgtacaaaaaagcaggctaagcttgtcgaccatggtagtcctatagtgaaaatgacaattacttataacaacaaattagtgtgcaatggtcatgaattctttccttctattgtcacttctagacctaatggtaacctttaatgtttaaccgttcacatttctaatatttacttatttgtaacatgtcgtcacgtgttagtttcattctttttatgaaccaaacatgcatgcaaagatatttttagatatttggacggcgagtgagatttgaaactaggaccgtttgcctgatacaatattaaaatatgtaaccattttatgtacaagtttaaactgttgatagtagcatattttttacttttatttaagtatactatattccaacaggtaagttaacttaggtctagaagtgacaatagaaggaaagaattcatgaccattgcacactaatttgttgttataagtaattgtcattttcactataggactaggcgcgcccgggcaattgacccagctttcttgtacaaagtggtgagctc